European Patent Application EP 4 516 892 A1, published March 5, 2025. Title: 药物组合物、巨球型菌及其应用. Applicant: 慕恩（广州）生物科技有限公司. The sequence listing filed with the application follows.

SEQUENCE LISTING (3 sequences)

SEQ ID NO: 1 - RNA, 1428 nt, Megasphaera sp.
  source 1..1428: mol_type = rRNA
cagtcgaacgagaggacatgggaagcttgcttctctatagaatcgagtggcaaacgggtgagtaacgcgtaagcaacctgccctgcagatggggacaacagctggaaacggctgctaataccgaatacgaagactgtgccgcatggtacggacttgaaaggatggcctctacattatgctatcgctgcaggaggggcttgcgtctgattagctagttggaggggtaacggcccaccaaggcgacgatcagtagccggtctgagaggatgaacggccacattgggactgagacacggcccagactcctacgggaggcagcagtggggaatcttccgcaatggacgaaagtctgacggagcaacgccgcgtgagtgatgacggccttcgggttgtaaaactctgttatacgggacgaatggacgagaggccaataccctttcggagtgacggtaccgtaagagaaagccacggctaactacgtgccagcagccgcggtaatacgtaggtggcaagcgttgtccggaattattgggcgtaaagggcgcgcaggtggtttcttaagtctgtcttaaaagtgcggggcttaaccccgtgaggggacggaaactgggagactagagtatcggagaggaaagcggaattcctagtgtagcggtgaaatgcgtagatattaggaggaacaccagtggcgaaagcggctttctggacgacaactgacactgaggcgcgaaagccaggggagcaaacgggattagataccccggtagtcctggccgtaaacgatgggtactaggtgtaggaggtaccacccccttctgtgccggagttaacgcaataagtaccccgcctggggagtacggccgcaaggctgaaactcaaaggaattgacgggggcccgcacaagcggtggagtatgtggtttaattcgacgcaacgcgaagaaccttaccaagccttgacattgatcgcaagggaaagagatttcctgttcctcttcggaggacgagaaaacaggtggtgcacggctgtcgtcagctcgtgtcgtgagatgttgggttaagtcccgcaacgagcgcaacccctatcttctgttaccagcacgtgatggtggggactcaggagagactgccgcagacaatgcggaggaaggcggggatgacgtcaagtcatcatgccccttatggcttgggctacacacgtactacaatggctcttaatagagggaagcgaaagggcgacctggagcaaaccccaaaaacagagtctcagttcggattgcaggctgcaactcgcctgcatgaaggaggaatcgctagtaatcgcaggtcagcatactgcggtgaatacgttcccgggccttgtacacaccgcccgtcacaccacgaaagtcattcacacccgaagccggtgaggcaaccgcaaggaacc

SEQ ID NO: 2 - RNA, 1443 nt, Megasphaera sp.
  source 1..1443: mol_type = rRNA
taccatgcagtcgaacgggaggacatgggaagcttgcttcctatggactctagtggcaaacgggtgagtaacgcgtaagcaacctgccctccggatggggacaacagctggaaacggctgctaataccgaatacgtttccattgccgcatggcagtgggaagaaaggtggcctctgaatatgctaccgccgggggaggggcttgcgtctgattagctagttggaggggtaacggcccaccaaggcgacgatcagtagccggtctgagaggatgaacggccacattggaactgagacacggtccagactcctacgggaggcagcagtggggaatcttccgcaatgggcgaaagcctgacggagcaacgccgcgtgagcgaagacggccttcgggttgtaaagctctgttatacgggacgaacggctagtgtgccaataccacattagaatgacggtaccgtaagagaaagccacggctaactacgtgccagcagccgcggtaatacgtaggtggcaagcgttgtccggaattattgggcgtaaagggcgcgcaggcggtttcataagtctgtcttaaaagtgcggggcttaaccccgtgaggggacggaaactgtgagactggagtgtcggagagaaagcggaattcctagtgtagcggtgaaatgcgtagatattaggaggaacaccagtggcgaaagcggctttctggacgacaactgacgctgaggcgcgaaagccaggggagcgaacgggattagataccccggtagtcctggccgtaaacgatggatactaggtgtagggggtatcgacccctcctgtgccggagttaacgcaataagtatcccgcctggggagtacggccgcaaggctgaaactcaaaggaattgacgggggcccgcacaagcggtggagtatgtggtttaattcgacgcaacgcgaagaaccttaccaagccttgacattgagtgctatctccagagatggagagttcttcttcggaagacgcgaaaacaggtggtgcacggctgtcgtcagctcgtgtcgtgagatgttgggttaagtcccgcaacgagcgcaacccctatcttctgttgccagcgcgtcatggcggggactcaggagagactgccgcagacaatgcggaggaaggcggggatgacgtcaagtcatcatgccccttatggcttgggctacacacgtactacaatggctcttaatagagggaagcgaaggagcgatccggagcaaaccccaaaaacagagtcccagttcggattgcaggctgcaacccgcctgcatgaagcaggaatcgctagtaatcgcaggtcagcatactgcggtgaatacgttcccgggccttgtacacaccgcccgtcacaccacgaaagtcattcacacccgaagccggtgaggtaaccgttacggagccagccgtcgaag

SEQ ID NO: 3 - RNA, 1404 nt, Megasphaera sp.
  source 1..1404: mol_type = rRNA
agtcgaacgggaggacatgggaagcttgcttcctatggactctagtggcaaacgggtgagtaacgcgtaagcaacctgccctccggatggggacaacagctggaaacggctgctaataccgaatgcgttttagctgtcgcatgatagtgaaaagaaaggtggcctctgaatatgctaccgccgggggaggggcttgcgtctgattagctagttggaggggtaacggcccaccaaggcgacgatcagtagccggtctgagaggatgaacggccacattggaactgagacacggtccagactcctacgggaggcagcagtggggaatcttccgcaatgggcgaaagcctgacggagcaacgccgcgtgagcgaagacggccttcgggttgtaaagctctgttatacgggacgaacggctagtgtgccaataccacattagaatgacggtaccgtaagaaaaagccacggctaactacgtgccagcagccgcggtaatacgtaggtggcaagcgttgtccggaattattgggcgtaaagggcgcgcaagcggtttcataagtctgtcttaaaagtgcggggcttaaccccgtgaggggacggaaactgtgagactggagtgtcggagaggaaagcggaattcctagtgtagcggtgaaatgcgtagatattaggaggaacaccagtggcgaaagcggctttctggacgacaactgacgctgaggcgcgaaagccaggggagcgaacgggattaaaaacccccgtaatcctgggcctaaacgatgggtactaggtgtagggggtatcgacccctcctgtgccggagttaacgcaataagtatcccgcctggggagtacggccgcaaggctgaaactcaaaggaattgacgggggcccgcacaagcggtggagtatgtggtttaattcgacgcaacgcgaagaaccttaccaagccttgacattgagtgctatctccagagatggggagttcttcttcggaggacgcgaaaacaggtggtgcacggctgtcgtcagctcgtgtcgtgagatgttgggttaagtcccgcaacgagcgcaacccctatcttctgttgccagcgcgtcatggtggggactcaggagagactgccgcagacaatgcggaggaaggcggggatgacgtcaagtcatcatgccccttatggcttgggctacacacgtactacaatggctcttaatagagggaagcgaaggagcgatccggagcaaaccccaaaaacagagtcccagttcggattgcaggctgcaacccgcctgcatgaagcaggaatcgctagtaatcgcaggtcagcatactgcggtgaatacgttcccgggccttgtacacaccgcccgtcacaccacgaaagtcattcacacccgaagccgg